European Patent Specification EP 3 337 893 B1, published July 19, 2023. Title: INCREASING PRODUCTIVITY OF E. COLI HOST CELLS THAT FUNCTIONALLY EXPRESS P450 ENZYMES. Applicant: Manus Biosynthesis MAK, Huey-Ming TIBREWALA, Srishti DONAL, Jason LI, Liwei PIRIE, Christopher KUMARAN, Ajikumar Parayil. The sequence listing filed with the application follows.

SEQUENCE LISTING (60 sequences)

SEQ ID NO: 1 - protein, 513 aa, Zingiber zerumbet
MEAISLFSPFFFITLFLGFFITLLIKRSSRSSVHKQQVLLASLPPSPPRLPLIGNIHQLVGGNPHRILLQLARTHGPLICLRLGQVDQVVASSVEAVEEIIKRHDLKFADRPRDLTFSRIFFYDGNAVVMTPYGGEWKQMRKIYAMELLNSRRVKSFAAIREDVARKLTGEIAHKAFAQTPVINLSEMVMSMINAIVIRVAFGDKCKQQAYFLHLVKEAMSYVSSFSVADMYPSLKFLDTLTGLKSKLEGVHGKLDKVFDEIIAQRQAALAAEQAEEDLIIDVLLKLKDEGNQEFPITYTSVKAIVMEIFLAGTETSSSVIDWVMSELIKNPKAMEKVQKEMREAMQGKTKLEESDIPKFSYLNLVIKETLRLHPPGPLLFPRECRETCEVMGYRVPAGARLLINAFALSRDEKYWGSDAESFKPERFEGISVDFKGSNFEFMPFGAGRRICPGMTFGISSVEVALAHLLFHFDWQLPQGMKIEDLDMMEVSGMSATRRSPLLVLAKLIIPLP

SEQ ID NO: 2 - protein, 496 aa, Barnadesia spinosa
MELTLTTSLGLAVFVFILFKLLTGSKSTKNSLPEAWRLPIIGHMHHLVGTLPHRGVTDMARKYGSLMHLQLGEVSTIVVSSPRWAKEVLTTYDITFANRPETLTGEIVAYHNTDIVLSPYGEYWRQLRKLCTLELLSAKKVKSFQSLREEECWNLVKEVRSSGSGSPVDLSESIFKLIATILSRAAFGKGIKDQREFTEIVKEILRLTGGFDVADIFPSKKILHHLSGKRAKLTNIHNKLDSLINNIVSEHPGSRTSSSQESLLDVLLRLKDSAELPLTSDNVKAVILDMFGAGTDTSSATIEWAISELIRCPRAMEKVQTELRQALNGKERIQEEDIQELSYLKLVIKETLRLHPPLPLVMPRECREPCVLAGYEIPTKTKLIVNVFAINRDPEYWKDAETFMPERFENSPINIMGSEYEYLPFGAGRRMCPGAALGLANVELPLAHILYYFNWKLPNGARLDELDMSECFGATVQRKSELLLVPTAYKTANNSA

SEQ ID NO: 3 - protein, 502 aa, Hyoscyamus muticus
MQFFSLVSIFLFLSFLFLLRKWKNSNSQSKKLPPGPWKLPLLGSMLHMVGGLPHHVLRDLAKKYGPLMHLQLGEVSAVVVTSPDMAKEVLKTHDIAFASRPKLLAPEIVCYNRSDIAFCPYGDYWRQMRKICVLEVLSAKNVRSFSSIRRDEVLRLVNFVRSSTSEPVNFTERLFLFTSSMTCRSAFGKVFKEQETFIQLIKEVIGLAGGFDVADIFPSLKFLHVLTGMEGKIMKAHHKVDAIVEDVINEHKKNLAMGKTNGALGGEDLIDVLLRLMNDGGLQFPITNDNIKAIIFDMFAAGTETSSSTLVWAMVQMMRNPTILAKAQAEVREAFKGKETFDENDVEELKYLKLVIKETLRLHPPVPLLVPRECREETEINGYTIPVKTKVMVNVWALGRDPKYWDDADNFKPERFEQCSVDFIGNNFEYLPFGGGRRICPGISFGLANVYLPLAQLLYHFDWKLPTGMEPKDLDLTELVGVTAARKSDLMLVATPYQPSRE

SEQ ID NO: 4 - protein, 488 aa, Lactuca sativa
MELSITTSIALATIVFFLYKLATRPKSTKKQLPEASRLPIIGHMHHLIGTMPHRGVMDLARKHGSLMHLQLGEVSTIVVSSPKWAKEILTTYDITFANRPETLTGEIIAYHNTDIVLAPYGEYWRQLRKLCTLELLSVKKVKSFQSIREEECWNLVKEVKESGSGKPINLSESIFTMIATILSRAAFGKGIKDQREFTEIVKEILRQTGGFDVADIFPSKKFLHHLSGKRARLTSIHKKLDNLINNIVAEHHVSTSSKANETLLDVLLRLKDSAEFPLTADNVKAIILDMFGAGTDTSSATVEWAISELIRCPRAMEKVQAELRQALNGKEKIQEEDIQDLAYLNLVIRETLRLHPPLPLVMPRECREPVNLAGYEIANKTKLIVNVFAINRDPEYWKDAEAFIPERFENNPNNIMGADYEYLPFGAGRRMCPGAALGLANVQLPLANILYHFNWKLPNGASHDQLDMTESFGATVQRKTELLLVPSF

SEQ ID NO: 5 - protein, 504 aa, Nicotiani tabacum
MQFFSLVSIFLFLSFLFLLRKWKNSNSQSKKLPPGPWKIPILGSMLHMIGGEPHHVLRDLAKKYGPLMHLQLGEISAVVVTSRDMAKEVLKTHDVVFASRPKIVAMDIICYNQSDIAFSPYGDHWRQMRKICVMELLNAKNVRSFSSIRRDEVVRLIDSIRSDSSSGELVNFTQRIIWFASSMTCRSAFGQVLKGQDIFAKKIREVIGLAEGFDVVDIFPTYKFLHVLSGMKRKLLNAHLKVDAIVEDVINEHKKNLAAGKSNGALGGEDLIDVLLRLMNDTSLQFPITNDNIKAVIVDMFAAGTETSSTTTVWAMAEMMKNPSVFTKAQAEVREAFRDKVSFDENDVEELKYLKLVIKETLRLHPPSPLLVPRECREDTDINGYTIPAKTKVMVNVWALGRDPKYWDDAESFKPERFEQCSVDFFGNNFEFLPFGGGRRICPGMSFGLANLYLPLAQLLYHFDWKLPTGIMPRDLDLTELSGITIARKGGLYLNATPYQPSRE

SEQ ID NO: 6 - protein, 522 aa, Citrus x paradisi
MELPLKSIALTIVIVTVLTWAWRVLNWVWLRPKKLEKFLRQQGLKGNSYRLLFGDLKENSIELKEAKARPLSLDDDIAIRVNPFLHKLVNDYGKNSFMWFGPTPRVNIMNPDQIKAIFTKINDFQKVNSIPLARLLIVGLATLEGEKWAKHRKLINPAFHQEKLKLMLPAFYLSCIEIITKWEKQMSVEGSSELDVWPYLANLTSDVISRTAFGSSYEEGRRIFQLQAELAELTMQVFRSVHIPGWRFLPTKRNRRMKEIDKEIRASLMGIIKNREKAMRAGEAANNDLLGILMETSFREIEEHGNNKNVGFSMNDVIEECKLFYFAGQETTSVLLNWTMVLLSKHQDWQERARQEVLQVFGNNKPDYDGLNHLKIVQMILYEVLRLYPPVTVLSRAVFKETKLGNLTLPAGVQIGLPMILVHQDPELWGDDAVEFKPERFAEGISKAAKNQVSYFPFALGPRICVGQNFALVEAKMATAMILQNYSFELSPSYVHAPTAVPTLHPELGTQLILRKLWCKNN

SEQ ID NO: 7 - protein, 495 aa, Artemesia annua
MKSILKAMALSLTTSIALATILLFVYKFATRSKSTKKSLPEPWRLPIIGHMHHLIGTTPHRGVRDLARKYGSLMHLQLGEVPTIVVSSPKWAKEILTTYDITFANRPETLTGEIVLYHNTDVVLAPYGEYWRQLRKICTLELLSVKKVKSFQSLREEECWNLVQEIKASGSGRPVNLSENVFKLIATILSRAAFGKGIKDQKELTEIVKEILRQTGGFDVADIFPSKKFLHHLSGKRARLTSLRKKIDNLIDNLVAEHTVNTSSKTNETLLDVLLRLKDSAEFPLTSDNIKAIILDMFGAGTDTSSSTIEWAISELIKCPKAMEKVQAELRKALNGKEKIHEEDIQELSYLNMVIKETLRLHPPLPLVLPRECRQPVNLAGYNIPNKTKLIVNVFAINRDPEYWKDAEAFIPERFENSSATVMGAEYEYLPFGAGRRMCPGAALGLANVQLPLANILYHFNWKLPNGVSYDQIDMTESSGATMQRKTELLLVPSF

SEQ ID NO: 8 - protein, 509 aa, Arabidopsis thaliana
MAFFSMISILLGFVISSFIFIFFFKKLLSFSRKNMSEVSTLPSVPVVPGFPVIGNLLQLKEKKPHKTFTRWSEIYGPIYSIKMGSSSLIVLNSTETAKEAMVTRFSSISTRKLSNALTVLTCDKSMVATSDYDDFHKLVKRCLLNGLLGANAQKRKRHYRDALIENVSSKLHAHARDHPQEPVNFRAIFEHELFGVALKQAFGKDVESIYVKELGVTLSKDEIFKVLVHDMMEGAIDVDWRDFFPYLKWIPNKSFEARIQQKHKRRLAVMNALIQDRLKQNGSESDDDCYLNFLMSEAKTLTKEQIAILVWETIIETADTTLVTTEWAIYELAKHPSVQDRLCKEIQNVCGGEKFKEEQLSQVPYLNGVFHETLRKYSPAPLVPIRYAHEDTQIGGYHVPAGSEIAINIYGCNMDKKRWERPEDWWPERFLDDGKYETSDLHKTMAFGAGKRVCAGALQASLMAGIAIGRLVQEFEWKLRDGEEENVDTYGLTSQKLYPLMAIINPRRS

SEQ ID NO: 9 - protein, 513 aa, Stevia rebaudiana
MDAVTGLLTVPATAITIGGTAVALAVALIFWYLKSYTSARRSQSNHLPRVPEVPGVPLLGNLLQLKEKKPYMTFTRWAATYGPIYSIKTGATSMVVVSSNEIAKEALVTRFQSISTRNLSKALKVLTADKTMVAMSDYDDYHKTVKRHILTAVLGPNAQKKHRIHRDIMMDNISTQLHEFVKNNPEQEEVDLRKIFQSELFGLAMRQALGKDVESLYVEDLKITMNRDEIFQVLVVDPMMGAIDVDWRDFFPYLKWVPNKKFENTIQQMYIRREAVMKSLIKEHKKRIASGEKLNSYIDYLLSEAQTLTDQQLLMSLWEPIIESSDTTMVTTEWAMYELAKNPKLQDRLYRDIKSVCGSEKITEEHLSQLPYITAIFHETLRRHSPVPIIPLRHVHEDTVLGGYHVPAGTELAVNIYGCNMDKNVWENPEEWNPERFMKENETIDFQKTMAFGGGKRVCAGSLQALLTASIGIGRMVQEFEWKLKDMTQEEVNTIGLTTQMLRPLRAIIKPRI

SEQ ID NO: 10 - protein, 546 aa, Physcomitrella patens
MAKHLATQLLQQWNEALKTMPPGFRTAGKILVWEELASNKVLITIALAWVLLFVARTCLRNKKRLPPAIPGGLPVLGNLLQLTEKKPHRTFTAWSKEHGPIFTIKVGSVPQAVVNNSEIAKEVLVTKFASISKRQMPMALRVLTRDKTMVAMSDYGEEHRMLKKLVMTNLLGPTTQNKNRSLRDDALIGMIEGVLAELKASPTSPKVVNVRDYVQRSLFPFALQQVFGYIPDQVEVLELGTCVSTWDMFDALVVAPLSAVINVDWRDFFPALRWIPNRSVEDLVRTVDFKRNSIMKALIRAQRMRLANLKEPPRCYADIALTEATHLTEKQLEMSLWEPIIESADTTLVTSEWAMYEIAKNPDCQDRLYREIVSVAGTERMVTEDDLPNMPYLGAIIKETLRKYTPVPLIPSRFVEEDITLGGYDIPKGYQILVNLFAIANDPAVWSNPEKWDPERMLANKKVDMGFRDFSLMPFGAGKRMCAGITQAMFIIPMNVAALVQHCEWRLSPQEISNINNKIEDVVYLTTHKLSPLSCEATPRISHRLP

SEQ ID NO: 11 - protein, 1049 aa, Bacillus megaterium
MTIKEMPQPKTFGELKNLPLLNTDKPVQALMKIADELGEIFKFEAPGRVTRYLSSQRLIKEACDESRFDKNLSQALKFVRDFAGDGLATSWTHEKNWKKAHNILLPSFSQQAMKGYHAMMVDIAVQLVQKWERLNADEHIEVPEDMTRLTLDTIGLCGFNYRFNSFYRDQPHPFITSMVRALDEAMNKLQRANPDDPAYDENKRQFQEDIKVMNDLVDKIIADRKASGEQSDDLLTHMLNGKDPETGEPLDDENIRYQIITFLIAGHETTSGLLSFALYFLVKNPHVLQKAAEEAARVLVDPVPSYKQVKQLKYVGMVLNEALRLWPTIPAFSLYAKEDTVLGGEYPLEKGDELMVLIPQLHRDKTIWGDDVEEFRPERFENPSAIPQHAFKPFGNGQRACIGQQFALHEATLVLGMMLKHFDFEDHTNYELDIKETLTLKPEGFVVKAKSKKIPLGGIPSPSTEQSAKKVRKKAENAHNTPLLVLYGSNMGTAEGTARDLADIAMSKGFAPQVATLDSHAGNLPREGAVLIVTASYNGHPPDNAKQFVDWLDQASADEVKGVRYSVFGCGDKNWATTYQKVPAFIDETLAAKGAENIADRGEADASDDFEGTYEEWREHMWSDVAAYFNLDIENSEDNKSTLSLQFVDSAADMPLAKMHGAFSTNVVASKELQQPGSARSTRHLEIELPKEASYQEGDHLGVIPRNYEGIVNRVTARFGLDASQQIRLEAEEEKLAHLPLAKTVSVEELLQYVELQDPVTRTQLRAMAAKTVCPPHKVELEALLEKQAYKEQVLAKRLTMLELLEKYPACEMKFSEFIALLPSIRPRYYSISSSPRVDEKQASITVSVVSGEAWSGYGEYKGIASNYLAELQEGDTITCFISTPQSEFTLPKDPETPLIMVGPGTGVAPFRGFVQARKQLKEQGQSLGEAHLYFGCRSPHEDYLYQEELENAQSEGIITLHTAFSRMPNQPKTYVQHVMEQDGKKLIELLDQGAHFYICGDGSQMAPAVEATLMKSYADVHQVSEADARLWLQQLEEKGRYAKDVWAG

SEQ ID NO: 12 - protein, 396 aa, Pleurotus sapidus
MRYGCAAVALFYLTAMGKLHPLAIIPDYKGSMAASVTIFNKRTNPLDISVNQANDWPWRYAKTCVLSSDWALHEMIIHLNNTHLVEEAVIVAAQRKLSPSHIVFRLLEPHWVVTLSLNALARSVLIPEVIVPIAGFSAPHIFQFIRESFTNFDWKSLYVPADLESRGFPVDQLNSPKFHNYAYARDINDMWTTLKKFVSSVLQDAQYYPDDASVAGDTQIQAWCDEMRSGMGAGMTNFPESITTVDDLVNMVTMCIHIAAPQHTAVNYLQQYYQTFVSNKPSALFSPLPTSIAQLQKYTESDLMAALPLNAKRQWLLMAQIPYLLSMQVQEDENIVTYAANASTDKDPIIASAGRQLAADLKKLAAVFLVNSAQLDDQNTPYDVLAPEQLANAIVI

SEQ ID NO: 13 - protein, 640 aa, Pleurotus ostreatus
MAPTMSLSRSALKNVHLPYMVQHPEPTDCSTAMKHAAEGYDRARQMIAFLFDILDYESSVPQKFTPEEKKEKYTWSHSDKFPPHLAIIPEDIDVPAYIIFSIVRLVQTLSIMSGIQCNERLAPGPEQNTMEKLTKWNAERHKNQGWVKDMFNEPNIGLRNDWYTDAVFAQQFFTGPNPTTITLASDTWMKAFTEEAASQGKRDLISLFRSAPPNSFYVQDFSDFRARMGAKPDEELCATSDGGVTRYGCAAVALFYLPPTGELHPLAIVPDYKGSMAASITLFNKRVDPSDASVDQANDWPWRYAKTCVLSADWVLHEMIIHLNNTHLVQEAVIVAVQRTLPDSHIVFRLLKPHWVVTLSLNAQARSVLIPEVIVPIAGFSELRIFQFVGHAFTNFDWKALYVPTDLEFRGFPLDRLDDDKFHNYAYAKDIKDMWMALRKFVSSVLKDGKYYPDDSAVAADAQIQDWCDEMRSEKGAGMKKFPESISTLDDLIDMVTMCIHIAAPQHTAVNYLQQYYQTFVPNKPSALFSPLPTLLSQLESYTESDLMAALPLGAKQEWLLMAQVPYLLSKEVEQDGNIVTYAGTASNNEDPIIAAAGKELSADLVILAGVFLKNSEKLDDQNTAYNVLAPDQLANAIVI

SEQ ID NO: 14 - protein, 495 aa, Cichorium intybus
MEISIPTTLGLAVIIFIIFKLLTRTTSKKNLLPEPWRLPIIGHMHHLIGTMPHRGVMELARKHGSLMHLQLGEVSTIVVSSPRWAKEVLTTYDITFANRPETLTGEIVAYHNTDIVLAPYGEYWRQLRKLCTLELLSNKKVKSFQSLREEECWNLVKDIRSTGQGSPINLSENIFKMIATILSRAAFGKGIKDQMKFTELVKEILRLTGGFDVADIFPSKKLLHHLSGKRAKLTNIHNKLDNLINNIIAEHPGNRTSSSQETLLDVLLRLKESAEFPLTADNVKAVILDMFGAGTDTSSATIEWAISELIRCPRAMEKVQTELRQALNGKERIQEEDLQELNYLKLVIKETLRLHPPLPLVMPRECREPCVLGGYDIPSKTKLIVNVFAINRDPEYWKDAETFMPERFENSPITVMGSEYEYLPFGAGRRMCPGAALGLANVELPLAHILYFNWKLPNGKTFEDLDMTESFGATVQRKTELLLVPTDFQTLTAST

SEQ ID NO: 15 - protein, 488 aa, Helianthus annuus
MEVSLTTSIALATIVFFLYKLLTRPTSSKNRLPEPWRLPIIGHMHHLIGTMPHRGVMDLARKYGSLMHLQLGEVSAIVVSSPKWAKEILTTYDIPFANRPETLTGEIIAYHNTDIVLAPYGEYWRQLRKLCTLELLSVKKVKSFQSLREEECWNLVQEIKASGSGTPFNLSEGIFKVIATVLSRAAFGKGIKDQKQFTEIVKEILRETGGFDVADIFPSKKFLHHLSGKRGRLTSIHNKLDSLINNLVAEHTVSKSSKVNETLLDVLLRLKNSEEFPLTADNVKAIILDMFGAGTDTSSATVEWAISELIRCPRAMEKVQAELRQALNGKERIKEEEIQDLPYLNLVIRETLRLHPPLPLVMPRECRQAMNLAGYDVANKTKLIVNVFAINRDPEYWKDAESFNPERFENSNTTIMGADYEYLPFGAGRRMCPGSALGLANVQLPLANILYYFKWKLPNGASHDQLDMTESFGATVQRKTELMLVPSF

SEQ ID NO: 16 - protein, 425 aa, Escherichia coli
MLELLYTALLYLIQPLIWIRLWVRGRKAPAYRKRWGERYGFYRHPLKPGGIMLHSVSVGETLAAIPLVRALRHRYPDLPITVTTMTPTGSERVQSAFGKDVQHVYLPYDLPDALNRFLNKVDPKLVLIMETELWPNLIAALHKRKIPLVIANARLSARSAAGYAKLGKFVRRLLRRITLIAAQNEEDGARFVALGAKNNQVTVTGSLKFDISVTPQLAAKAVTLRRQWAPHRPVWIATSTHEGEESVVIAAHQALLQQFPNLLLILVPRHPERFPDAINLVRQAGLSYITRSSGEVPSTSTQVVVGDTMGELMLLYGIADLAFVGGSLVERGGHNPLEAAAHAIPVLMGPHTFNFKDICARLEQASGLITVTDATTLAKEVSSLLTDADYRSFYGRHAVEVLYQNQGALQRLLQLLEPYLPPKTH

SEQ ID NO: 17 - protein, 66 aa, Escherichia coli
MDWLAKYWWILVIVFLVGVLLNVIKDLKRVDHKKFLANKPELPPHRDFNDKWDDDDDWPKKDQPKK

SEQ ID NO: 18 - protein, 132 aa, Escherichia coli
MTWEYALIGLVVGIIIGAVAMRFGNRKLRQQQALQYELEKNKAELDEYREELVSHFARSAELLDTMAHDYRQLYQHMAKSSSSLLPELSAEANPFRNRLAESEASNDQAPVQMPRDYSEGASGLLRTGAKRD

SEQ ID NO: 19 - protein, 294 aa, Escherichia coli
MKPFLRWCFVATALTLAGCSNTSWRKSEVLAVPLQPTLQQEVILARMEQILASRALTDDERAQLLYERGVLYDSLGLRALARNDFSQALAIRPDMPEVFNYLGIYLTQAGNFDAAYEAFDSVLELDPTYNYAHLNRGIALYYGGRDKLAQDDLLAFYQDDPNDPFRSLWLYLAEQKLDEKQAKEVLKQHFEKSDKEQWGWNIVEFYLGNISEQTLMERLKADATDNTSLAEHLSETNFYLGKYYLSLGDLDSATALFKLAVANNVHNFVEHRYALLELSLLGQDQDDLAESDQQ

SEQ ID NO: 20 - protein, 119 aa, Escherichia coli
MSKPPLFFIVIIGLIVVAASFRFMQQRREKADNDMAPLQQKLVVVSNKREKPINDRRSRQQEVTPAGTSIRYEASFKPQSGGMEQTFRLDAQQYHALTVGDKGTLSYKGTRFVSFVGEQ

SEQ ID NO: 21 - protein, 328 aa, Escherichia coli
MMQDLRLILIIVGAIAIIALLVHGFWTSRKERSSMFRDRPLKRMKSKRDDDSYDEDVEDDEGVGEVRVHRVNHAPANAQEHEAARPSPQHQYQPPYASAQPRQPVQQPPEAQVPPQHAPHPAQPVQQPAYQPQPEQPLQQPVSPQVAPAPQPVHSAPQPAQQAFQPAEPVAAPQPEPVAEPAPVMDKPKRKEAVIIMNVAAHHGSELNGELLLNSIQQAGFIFGDMNIYHRHLSPDGSGPALFSLANMVKPGTFDPEMKDFTTPGVTIFMQVPSYGDELQNFKLMLQSAQHIADEVGGVVLDDQRRMMTPQKLREYQDIIREVKDANA

SEQ ID NO: 22 - protein, 507 aa, Escherichia coli
MRNTLIPILVAICLFITGVAILNIQLWYSAKAEYLAGARYAANNINHILEEASQATQTAVNIAGKECNLEEQYQLGTEAALKPHLRTIIILKQGIVWCTSLPGNRVLLSRIPVFPDSNLLLAPAIDTVNRLPILLYQNQFADTRILVTISDQHIRGALNVPLKGVRYVLRVADDIIGPTGDVMTLNGHYPYTEKVHSTKYHFTIIFNPPPLFSFYRLIDKGFGILIFILLIACAAAFLLDRYFNKSATPEEILRRAINNGEIVPFYQPVVNGREGTLRGVEVLARWKQPHGGYISPAAFIPLAEKSGLIVPLTQSLMNQVARQMNAIASKLPEGFHIGINFSASHIISPTFVDECLNFRDSFTRRDLNLVLEVTEREPLNVDESLVQRLNILHENGFVIALDDFGTGYSGLSYLHDLHIDYIKIDHSFVGRVNADPESTRILDCVLDLARKLSISIVAEGVETKEQLDYLNQNYITFQQGYYFYKPVTYIDLVKIILSKPKVKVVVE

SEQ ID NO: 23 - protein, 271 aa, Escherichia coli
MQYWGKIIGVAVALLMGGGFWGVVLGLLIGHMFDKARSRKMAWFANQRERQALFFATTFEVMGHLTKSKGRVTEADIHIASQLMDRMNLHGASRTAAQNAFRVGKSDNYPLREKMRQFRSVCFGRFDLIRMFLEIQIQAAFADGSLHPNERAVLYVIAEELGISRAQFDQFLRMMQGGAQFGGGYQQQTGGGNWQQAQRGPTLEDACNVLGVKPTDDATTIKRAYRKLMSEHHPDKLVAKGLPPEMMEMAKQKAQEIQQAYELIKQQKGFK

SEQ ID NO: 24 - protein, 349 aa, Escherichia coli
MELLSEYGLFLAKIVTVVLAIAAIAAIIVNVAQRNKRQRGELRVNNLSEQYKEMKEELAAALMDSHQQKQWHKAQKKKHKQEAKAAKAKAKLGEVATDSKPRVWVLDFKGSMDAHEVNSLREEITAVLAAFKPQDQVVLRLESPGGMVHGYGLAASQLQRLRDKNIPLTVTVDKVAASGGYMMACVADKIVSAPFAIVGSIGVVAQMPNFNRFLKSKDIDIELHTAGQYKRTLTLLGENTEEGREKFREELNETHQLFKDFVKRMRPSLDIEQVATGEHWYGQQAVEKGLVDEINTSDEVILSLMEGREVVNVRYMQRKRLIDRFTGSAAESADRLLLRWWQRGQKPLM

SEQ ID NO: 25 - protein, 328 aa, Escherichia coli
MIEKIWSGESPLWRLLLPLSWLYGLVSGAIRLCYKLKLKRAWRAPVPVVVVGNLTAGGNGKTPVVVWLVEQLQQRGIRVGVVSRGYGGKAESYPLLLSADTTTAQAGDEPVLIYQRTDAPVAVSPVRSDAVKAILAQHPDVQIIVTDDGLQHYRLARDVEIVVIDGVRRFGNGWWLPAGPMRERAGRLKSVDAVIVNGGVPRSGEIPMHLLPGQAVNLRTGTRCDVAQLEHVVAMAGIGHPPRFFATLKMCGVQPEKCVPLADHQSLNHADVSALVSAGQTLVMTEKDAVKCRAFAEENWWYLPVDAQLSGDEPAKLLTQLTLLASGN

SEQ ID NO: 26 - protein, 121 aa, Escherichia coli
MNNHATVQSSAPVSAAPLLQVSGALIAIIALILAAAWLVKRLGFAPKRTGVNGLKISASASLGARERVVVVDVEDARLVLGVTAGQINLLHKLPPSAPTEEIPQTDFQSVMKNLLKRSGRS

SEQ ID NO: 27 - protein, 295 aa, Escherichia coli
MLILLGYLVVLGTVFGGYLMTGGSLGALYQPAELVIIAGAGIGSFIVGNNGKAIKGTLKALPLLFRRSKYTKAMYMDLLALLYRLMAKSRQMGMFSLERDIENPRESEIFASYPRILADSVMLDFIVDYLRLIISGHMNTFEIEALMDEEIETHESEAEVPANSLALVGDSLPAFGIVAAVMGVVHALGSADRPAAELGALIAHAMVGTFLGILLAYGFISPLATVLRQKSAETSKMMQCVKVTLLSNLNGYAPPIAVEFGRKTLYSSERPSFIELEEHVRAVKNPQQQTTTEEA

SEQ ID NO: 28 - protein, 293 aa, Escherichia coli
MMRIALFLLTNLAVMVVFGLVLSLTGIQSSSVQGLMIMALLFGFGGSFVSLLMSKWMALRSVGGEVIEQPRNERERWLVNTVATQARQAGIAMPQVAIYHAPDINAFATGARRDASLVAVSTGLLQNMSPDEAEAVIAHEISHIANGDMVTMTLIQGVVNTFVIFISRILAQLAAGFMGGNRDEGEESNGNPLIYFAVATVLELVFGILASIITMWFSRHREFHADAGSAKLVGREKMIAALQRLKTSYEPQEATSMMALCINGKSKSLSELFMTHPPLDKRIEALRTGEYLK

SEQ ID NO: 29 - protein, 441 aa, Escherichia coli
MINRIVSFFILCLVLCIPLCVAYFHSGELMMRFVFFWPFFMSIMWIVGGVYFWVYRERHWPWGENAPAPQLKDNPSISIIIPCFNEEKNVEETIHAALAQRYENIEVIAVNDGSTDKTRAILDRMAAQIPHLRVIHLAQNQGKAIALKTGAAAAKSEYLVCIDGDALLDRDAAAYIVEPMLYNPRVGAVTGNPRIRTRSTLVGKIQVGEYSSIIGLIKRTQRIYGNVFTVSGVIAAFRRSALAEVGYWSDDMITEDIDISWKLQLNQWTIFYEPRALCWILMPETLKGLWKQRLRWAQGGAEVFLKNMTRLWRKENFRMWPLFFEYCLTTIWAFTCLVGFIIYAVQLAGVPLNIELTHIAATHTAGILLCTLCLLQFIVSLMIENRYEHNLTSSLFWIIWFPVIFWMLSLATTLVSFTRVMLMPKKQRARWVSPDRGILRG

SEQ ID NO: 30 - protein, 131 aa, Escherichia coli
MTSRFMLIFAAISGFIFVALGAFGAHVLSKTMGAVEMGWIQTGLEYQAFHTLAILGLAVAMQRRISIWFYWSSVFLALGTVLFSGSLYCLALSHLRLWAFVTPVGGVSFLAGWALMLVGAIRLKRKGVSHE

SEQ ID NO: 31 - protein, 655 aa, Escherichia coli
MNVIKTAICTLITLPVGLQAATSHSSSMTKDTITVVATGNQNTVFETPSMVSVVTNDTPWSKNAVTSAGMLRGVAGLSQTGAGRTNGQTFNLRGYDKSGVLVLVDGVRQLSDMAKSSGTYLDPALVKRIEVVRGPNSSLYGSGGLGGVVDFRTADAADFLPPGETNGVSLWGNIASGDHSTGSGLTWFGKTEKTDALLSVIMRKRGSIYQSDGERAPNKEKPAALFAKGSVSITDSNKAGASLRLYRNSTTEPGNPTLTHGDSGLRDRKTAQNDMQFWYQYAPADNSLINVKSTLYLSDITVKTNGHNKTAEWRNNRTSGVNVVNRSHSLIFPGAHQLSYGAEYYRQQQKPEGTATLYPEGHIDFTSLYFQDEMTMESYPVNIIVGSRYDRYNSFNARAGELNAERLSPRAAMSVSPTDWLMMYGSISSAFRAPTMAEMYRDDVHFYRKGKPNYWVPNLNLKPENNTTREIGAGIQLDSLLTDNDRLQLKGGYFGTDARNYIATRVDMKRMRSYSYNVSRARIWGWDIQGNYQSDYVDWMLSYNRTESMDASSREWLGSGNPDTLISDISIPVGHRGVYAGWRAELSAPATHVKKGDPCQDGYAIHSFSLSYKPVSVKGFEASVTLDNAFNKLAMNGKGVPLSGRTVNLYTRYQW

SEQ ID NO: 32 - protein, 102 aa, Escherichia coli
MKYLLIFLLVLAIFVISVTLGAQNDQQVTFNYLLAQGEYRISTLLAVLFAAGFAIGWLICGLFWLRVRVSLARAERKIKRLENQLSPATDVAVVPHSSAAKE

SEQ ID NO: 33 - protein, 710 aa, Stevia rebaudiana
MQSDSVKVSPFDLVSAAMNGKAMEKLNASESEDPTTLPALKMLVENRELLTLFTTSFAVLIGCLVFLMWRRSSSKKLVQDPVPQVIVVKKKEKESEVDDGKKKVSIFYGTQTGTAEGFAKALVEEAKVRYEKTSFKVIDLDDYAADDDEYEEKLKKESLAFFFLATYGDGEPTDNAANFYKWFTEGDDKGEWLKKLQYGVFGLGNRQYEHFNKIAIVVDDKLTEMGAKRLVPVGLGDDDQCIEDDFTAWKELVWPELDQLLRDEDDTSVTTPYTAAVLEYRVVYHDKPADSYAEDQTHTNGHVVHDAQHPSRSNVAFKKELHTSQSDRSCTHLEFDISHTGLSYETGDHVGVYSENLSEVVDEALKLLGLSPDTYFSVHADKEDGTPIGGASLPPPFPPCTLRDALTRYADVLSSPKKVALLALAAHASDPSEADRLKFLASPAGKDEYAQWIVANQRSLLEVMQSFPSAKPPLGVFFAAVAPRLQPRYYSISSSPKMSPNRIHVTCALVYETTPAGRIHRGLCSTWMKNAVPLTESPDCSQASIFVRTSNFRLPVDPKVPVIMIGPGTGLAPFRGFLQERLALKESGTELGSSIFFFGCRNRKVDFIYEDELNNFVETGALSELIVAFSREGTAKEYVQHKMSQKASDIWKLLSEGAYLYVCGDAKGMAKDVHRTLHTIVQEQGSLDSSKAELYVKNLQMSGRYLRDVW

SEQ ID NO: 34 - protein, 692 aa, Arabidopsis thaliana
MTSALYASDLFKQLKSIMGTDSLSDDVVLVIATTSLALVAGFVVLLWKKTTADRSGELKPLMIPKSLMAKDEDDDLDLGSGKTRVSIFFGTQTGTAEGFAKALSEEIKARYEKAAVKVIDLDDYAADDDQYEEKLKKETLAFFCVATYGDGEPTDNAARFSKWFTEENERDIKLQQLAYGVFALGNRQYEHFNKIGIVLDEELCKKGAKRLIEVGLGDDDQSIEDDFNAWKESLWSELDKLLKDEDDKSVATPYTAVIPEYRVVTHDPRFTTQKSMESNVANGNTTIDIHHPCRVDVAVQKELHTHESDRSCIHLEFDISRTGITYETGDHVGVYAENHVEIVEEAGKLLGHSLDLVFSIHADKEDGSPLESAVPPPFPGPCTLGTGLARYADLLNPPRKSALVALAAYATEPSEAEKLKHLTSPDGKDEYSQWIVASQRSLLEVMAAFPSAKPPLGVFFAAIAPRLQPRYYSISSCQDWAPSRVHVTSALVYGPTPTGRIHKGVCSTWMKNAVPAEKSHECSGAPIFIRASNFKLPSNPSTPIVMVGPGTGLAPFRGFLQERMALKEDGEELGSSLLFFGCRNRQMDFIYEDELNNFVDQGVISELIMAFSREGAQKEYVQHKMMEKAAQVWDLIKEEGYLYVCGDAKGMARDVHRTLHTIVQEQEGVSSSEAEAIVKKLQTEGRYLRDVW

SEQ ID NO: 35 - protein, 717 aa, Taxus cuspidata
MQANSNTVEGASQGKSLLDISRLDHIFALLLNGKGGDLGAMTGSALILTENSQNLMILTTALAVLVACVFFFVWRRGGSDTQKPAVRPTPLVKEEDEEEEDDSAKKKVTIFFGTQTGTAEGFAKALAEEAKARYEKAVFKVVDLDNYAADDEQYEEKLKKEKLAFFMLATYGDGEPTDNAARFYKWFLEGKEREPWLSDLTYGVFGLGNRQYEHFNKVAKAVDEVLIEQGAKRLVPVGLGDDDQCIEDDFTAWREQVWPELDQLLRDEDDEPTSATPYTAAIPEYRVEIYDSVVSVYEETHALKQNGQAVYDIHHPCRSNVAVRRELHTPLSDRSCIHLEFDISDTGLIYETGDHVGVHTENSIETVEEAAKLLGYQLDTIFSVHGDKEDGTPLGGSSLPPPFPGPCTLRTALARYADLLNPPRKAAFLALAAHASDPAEAERLKFLSSPAGKDEYSQWVTASQRSLLEIMAEFPSAKPPLGVFFAAIAPRLQPRYYSISSSPRFAPSRIHVTCALVYGPSPTGRIHKGVCSNWMKNSLPSEETHDCSWAPVFVRQSNFKLPADSTTPIVMVGPGTGFAPFRGFLQERAKLQEAGEKLGPAVLFFGCRNRQMDYIYEDELKGYVEKGILTNLIVAFSREGATKEYVQHKMLEKASDTWSLIAQGGYLYVCGDAKGMARDVHRTLHTIVQEQESVDSSKAEFLVKKLQMDGRYLRDIW

SEQ ID NO: 36 - protein, 705 aa, Artemesia annua
MAQSTTSVKLSPFDLMTALLNGKVSFDTSNTSDTNIPLAVFMENRELLMILTTSVAVLIGCVVVLVWRRSSSAAKKAAESPVIVVPKKVTEDEVDDGRKKVTVFFGTQTGTAEGFAKALVEEAKARYEKAVFKVIDLDDYAAEDDEYEEKLKKESLAFFFLATYGDGEPTDNAARFYKWFTEGEEKGEWLDKLQYAVFGLGNRQYEHFNKIAKVVDEKLVEQGAKRLVPVGMGDDDQCIEDDFTAWKELVWPELDQLLRDEDDTSVATPYTAAVAEYRVVFHDKPETYDQDQLTNGHAVHDAQHPCRSNVAVKKELHSPLSDRSCTHLEFDISNTGLSYETGDHVGVYVENLSEVVDEAEKLIGLPPHTYFSVHADNEDGTPLGGASLPPPFPPCTLRKALASYADVLSSPKKSALLALAAHATDSTEADRLKFLASPAGKDEYAQWIVASHRSLLEVMEAFPSAKPPLGVFFASVAPRLQPRYYSISSSPRFAPNRIHVTCALVYEQTPSGRVHKGVCSTWMKNAVPMTESQDCSWAPIYVRTSNFRLPSDPKVPVIMIGPGTGLAPFRGFLQERLAQKEAGTELGTAILFFGCRNRKVDFIYEDELNNFVETGALSELVTAFSREGATKEYVQHKMTQKASDIWNLLSEGAYLYVCGDAKGMAKDVHRTLHTIVQEQGSLDSSKAELYVKNLQMAGRYLRDVW

SEQ ID NO: 37 - protein, 693 aa, Arabidopsis thaliana
MATSALYASDLFKQLKSIMGTDSLSDDVVLVIATTSLALVAGFVVLLWKKTTADRSGELKPLMIPKSLMAKDEDDDLDLGSGKTRVSIFFGTQTGTAEGFAKALSEEIKARYEKAAVKVIDLDDYAADDDQYEEKLKKETLAFFCVATYGDGEPTDNAARFYKWFTEENERDIKLQQLAYGVFALGNRQYEHFNKIGIVLDEELCKKGAKRLIEVGLGDDDQSIEDDFNAWKESLWSELDKLLKDEDDKSVATPYTAVIPEYRVVTHDPRFTTQKSMESNVANGNTTIDIHHPCRVDVAVQKELHTHESDRSCIHLEFDISRTGITYETGDHVGVYAENHVEIVEEAGKLLGHSLDLVFSIHADKEDGSPLESAVPPPFPGPCTLGTGLARYADLLNPPRKSALVALAAYATEPSEAEKLKHLTSPDGKDEYSQWIVASQRSLLEVMAAFPSAKPPLGVFFAAIAPRLQPRYYSISSSPRLAPSRVHVTSALVYGPTPTGRIHKGVCSTWMKNAVPAEKSHECSGAPIFIRASNFKLPSNPSTPIVMVGPGTGLAPFRGFLQERMALKEDGEELGSSLLFFGCRNRQMDFIYEDELNNFVDQGVISELIMAFSREGAQKEYVQHKMMEKAAQVWDLIKEEGYLYVCGDAKGMARDVHRTLHTIVQEQEGVSSSEAEAIVKKLQTEGRYLRDVW

SEQ ID NO: 38 - protein, 712 aa, Arabidopsis thaliana
MASSSSSSSTSMIDLMAAIIKGEPVIVSDPANASAYESVAAELSSMLIENRQFAMIVTTSIAVLIGCIVMLVWRRSGSGNSKRVEPLKPLVIKPREEEIDDGRKKVTIFFGTQTGTAEGFAKALGEEAKARYEKTRFKIVDLDDYAADDDEYEEKLKKEDVAFFFLATYGDGEPTDNAARFYKWFTEGNDRGEWLKNLKYGVFGLGNRQYEHFNKVAKVVDDILVEQGAQRLVQVGLGDDDQCIEDDFTAWREALWPELDTILREEGDTAVATPYTAAVLEYRVSIHDSEDAKFNDINMANGNGYTVFDAQHPYKANVAVKRELHTPESDRSCIHLEFDIAGSGLTYETGDHVGVLCDNLSETVDEALRLLDMSPDTYFSLHAEKEDGTPISSSLPPPFPPCNLRTALTRYACLLSSPKKSALVALAAHASDPTEAERLKHLASPAGKDEYSKWVVESQRSLLEVMAEFPSAKPPLGVFFAGVAPRLQPRFYSISSSPKIAETRIHVTCALVYEKMPTGRIHKGVCSTWMKNAVPYEKSENCSSAPIFVRQSNFKLPSDSKVPIIMIGPGTGLAPFRGFLQERLALVESGVELGPSVLFFGCRNRRMDFIYEEELQRFVESGALAELSVAFSREGPTKEYVQHKMMDKASDIWNMISQGAYLYVCGDAKGMARDVHRSLHTIAQEQGSMDSTKAEGFVKNLQTSGRYLRDVW

SEQ ID NO: 39 - protein, 713 aa, Arabidopsis thaliana
MASSSSSSSTSMIDLMAAIIKGEPVIVSDPANASAYESVAAELSSMLIENRQFAMIVTTSIAVLIGCIVMLVWRRSGSGNSKRVEPLKPLVIKPREEEIDDGRKKVTIFFGTQTGTAEGFAKALGEEAKARYEKTRFKIVDLDDYAADDDEYEEKLKKEDVAFFFLATYGDGEPTDNAARFYKWFTEGNDRGEWLKNLKYGVFGLGNRQYEHFNKVAKVVDDILVEQGAQRLVQVGLGDDDQCIEDDFTAWREALWPELDTILREEGDTAVATPYTAAVLEYRVSIHDSEDAKFNDITLANGNGYTVFDAQHPYKANVAVKRELHTPESDRSCIHLEFDIAGSGLTMKLGDHVGVLCDNLSETVDEALRLLDMSPDTYFSLHAEKEDGTPISSSLPPPFPPCNLRTALTRYACLLSSPKKSALVALAAHASDPTEAERLKHLASPAGKDEYSKWVVESQRSLLEVMAEFPSAKPPLGVFFAGVAPRLQPRFYSISSSPKIAETRIHVTCALVYEKMPTGRIHKGVCSTWMKNAVPYEKSEKLFLGRPIFVRQSNFKLPSDSKVPIIMIGPGTGLAPFRGFLQERLALVESGVELGPSVLFFGCRNRRMDFIYEEELQRFVESGALAELSVAFSREGPTKEYVQHKMMDKASDIWNMISQGAYLYVCGDAKGMARDVHRSLHTIAQEQGSMDSTKAEGFVKNLQTSGRYLRDVW

SEQ ID NO: 40 - protein, 711 aa, Stevia rebaudiana
MAQSDSVKVSPFDLVSAAMNGKAMEKLNASESEDPTTLPALKMLVENRELLTLFTTSFAVLIGCLVFLMWRRSSSKKLVQDPVPQVIVVKKKEKESEVDDGKKKVSIFYGTQTGTAEGFAKALVEEAKVRYEKTSFKVIDLDDYAADDDEYEEKLKKESLAFFFLATYGDGEPTDNAANFYKWFTEGDDKGELLKKLQYGVFGLGNRQYEHFNKIAIVVDDKLTEMGAKRLVPVGLGDDDQCIEDDFTAWKELVWPELDQLLRDEDDTSVTTPYTAAVLEYRVVYHDKPADSYAEDQTHTNGHVVHDAQHPSRSNVAFKKELHTSQSDRSCTHLEFDISHTGLSYETGDHVGVYSENLSEVVDEALKLLGLSPDTYFSVHADKEDGTPIGGASLPPPFPPCTLRDALTRYADVLSSPKKVALLALAAHASDPSEADRLKFLASPAGKDEYAQWIVANQRSLLEVMQSFPSAKPPLGVFFAAVAPRLQPRYYSISSSPKMSPNRIHVTCALVYETTPAGRIHRGLCSTWMKNAVPLTESPDCSQASIFVRTSNFRLPVDPKVPVIMIGPGTGLAPFRGFLQERLALKESGTELGSSIFFFGCRNRKVDFIYEDELNNFVETGALSELIVAFSREGTAKEYVQHKMSQKASDIWKLLSEGAYLYVCGDAKGMAKDVHRTLHTIVQEQGSLDSSKAELYVKNLQMSGRYLRDVW

SEQ ID NO: 41 - protein, 710 aa, Stevia rebaudiana
MAQSESVEASTIDLMTAVLKDTVIDTANASDNGDSKMPPALAMMFEIRDLLLILTTSVAVLVGCFVVLVWKRSSGKKSGKELEPPKIVVPKRRLEQEVDDGKKKVTIFFGTQTGTAEGFAKALFEEAKARYEKAAFKVIDLDDYAADLDEYAEKLKKETYAFFFLATYGDGEPTDNAAKFYKWFTEGDEKGVWLQKLQYGVFGLGNRQYEHFNKIGIVVDDGLTEQGAKRIVPVGLGDDDQSIEDDFSAWKELVWPELDLLLRDEDDKAAATPYTAAIPEYRVVFHDKPDAFSDDHTQTNGHAVHDAQHPCRSNVAVKKELHTPESDRSCTHLEFDISHTGLSYETGDHVGVYCENLIEVVEEAGKLLGLSTDTYFSLHIDNEDGSPLGGPSLQPPFPPCTLRKALTNYADLLSSPKKSTLLALAAHASDPTEADRLRFLASREGKDEYAEWVVANQRSLLEVMEAFPSARPPLGVFFAAVAPRLQPRYYSISSSPKMEPNRIHVTCALVYEKTPAGRIHKGICSTWMKNAVPLTESQDCSWAPIFVRTSNFRLPIDPKVPVIMIGPGTGLAPFRGFLQERLALKESGTELGSSILFFGCRNRKVDYIYENELNNFVENGALSELDVAFSRDGPTKEYVQHKMTQKASEIWNMLSEGAYLYVCGDAKGMAKDVHRTLHTIVQEQGSLDSSKAELYVKNLQMSGRYLRDVW

SEQ ID NO: 42 - protein, 708 aa, Stevia rebaudiana
MAQSNSVKISPLDLVTALFSGKVLDTSNASESGESAMLPTIAMIMENRELLMILTTSVAVLIGCVVVLVWRRSSTKKSALEPPVIVVPKRVQEEEVDDGKKKVTVFFGTQTGTAEGFAKALVEEAKARYEKAVFKVIDLDDYAADDDEYEEKLKKESLAFFFLATYGDGEPTDNAARFYKWFTEGDAKGEWLNKLQYGVFGLGNRQYEHFNKIAKVVDDGLVEQGAKRLVPVGLGDDDQCIEDDFTAWKELVWPELDQLLRDEDDTTVATPYTAAVAEYRVVFHEKPDALSEDYSYTNGHAVHDAQHPCRSNVAVKKELHSPESDRSCTHLEFDISNTGLSYETGDHVGVYCENLSEVVNDAERLVGLPPDTYFSIHTDSEDGSPLGGASLPPPFPPCTLRKALTCYADVLSSPKKSALLALAAHATDPSEADRLKFLASPAGKDEYSQWIVASQRSLLEVMEAFPSAKPSLGVFFASVAPRLQPRYYSISSSPKMAPDRIHVTCALVYEKTPAGRIHKGVCSTWMKNAVPMTESQDCSWAPIYVRTSNFRLPSDPKVPVIMIGPGTGLAPFRGFLQERLALKEAGTDLGLSILFFGCRNRKVDFIYENELNNFVETGALSELIVAFSREGPTKEYVQHKMSEKASDIWNLLSEGAYLYVCGDAKGMAKDVHRTLHTIVQEQGSLDSSKAELYVKNLQMSGRYLRDVW

SEQ ID NO: 43 - protein, 706 aa, Pelargonium graveolens
MAQSSSGSMSPFDFMTAIIKGKMEPSNASLGAAGEVTAMILDNRELVMILTTSIAVLIGCVVVFIWRRSSSQTPTAVQPLKPLLAKETESEVDDGKQKVTIFFGTQTGTAEGFAKALADEAKARYDKVTFKVVDLDDYAADDEEYEEKLKKETLAFFFLATYGDGEPTDNAARFYKWFLEGKERGEWLQNLKFGVFGLGNRQYEHFNKIAIVVDEILAEQGGKRLISVGLGDDDQCIEDDFTAWRESLWPELDQLLRDEDDTTVSTPYTAAVLEYRVVFHDPADAPTLEKSYSNANGHSVVDAQHPLRANVAVRRELHTPASDRSCTHLEFDISGTGIAYETGDHVGVYCENLAETVEEALELLGLSPDTYFSVHADKEDGTPLSGSSLPPPFPPCTLRTALTLHADLLSSPKKSALLALAAHASDPTEADRLRHLASPAGKDEYAQWIVASQRSLLEVMAEFPSAKPPLGVFFASVAPRLQPRYYSISSSPRIAPSRIHVTCALVYEKTPTGRVHKGVCSTWMKNSVPSEKSDECSWAPIFVRQSNFKLPADAKVPIIMIGPGTGLAPFRGFLQERLALKEAGTELGPSILFFGCRNSKMDYIYEDELDNFVQNGALSELVLAFSREGPTKEYVQHKMMEKASDIWNLISQGAYLYVCGDAKGMARDVHRTLHTIAQEQGSLDSSKAESMVKNLQMSGRYLRDVW

SEQ ID NO: 44 - protein, 7 aa, Artificial sequence
  Synthetic sequence
GSGGGGS

SEQ ID NO: 45 - protein, 8 aa, Artificial sequence
  Synthetic sequence
GSGEAAAK

SEQ ID NO: 46 - protein, 13 aa, Artificial sequence
  Synthetic sequence
GSGEAAAKEAAAK

SEQ ID NO: 47 - protein, 9 aa, Artificial sequence
  Synthetic sequence
GSGMGSSSN

SEQ ID NO: 48 - protein, 491 aa, Zingiber zerumbet
LLIKRSSRSSVHKQQVLLASLPPSPPRLPLIGNIHQLVGGNPHRILLQLARTHGPLICLRLGQVDQVVASSVEAVEEIIKRHDLKFADRPRDLTFSRIFFYDGNAVVMTPYGGEWKQMRKIYAMELLNSRRVKSFAAIREDVARKLTGEIAHKAFAQTPVINLSEMVMSMINAIVIRVAFGDKCKQQAYFLHLVKEAMSYVSSFSVADMYPSLKFLDTLTGLKSKLEGVHGKLDKVFDEIIAQRQAALAAEQAEEDLIIDVLLKLKDEGNQEFPITYTSVKAIVMEIFLAGTETSSSVIDWVMSELIKNPKAMEKVQKEMREAMQGKTKLEESDIPKFSYLNLVIKETLRLHPPGPLLFPRECRETCEVMGYRVPAGARLLINAFALSRDEKYWGSDAESFKPERFEGISVDFKGSNFEFMPFGAGRRICPGMTFGISSVEVALAHLLFHFDWQLPQGMKIEDLDMMEVSGMSATRRSPLLVLAKLIIPLP

SEQ ID NO: 49 - protein, 476 aa, Barnadesia spinosa
LLTGSKSTKNSLPEAWRLPIIGHMHHLVGTLPHRGVTDMARKYGSLMHLQLGEVSTIVVSSPRWAKEVLTTYDITFANRPETLTGEIVAYHNTDIVLSPYGEYWRQLRKLCTLELLSAKKVKSFQSLREEECWNLVKEVRSSGSGSPVDLSESIFKLIATILSRAAFGKGIKDQREFTEIVKEILRLTGGFDVADIFPSKKILHHLSGKRAKLTNIHNKLDSLINNIVSEHPGSRTSSSQESLLDVLLRLKDSAELPLTSDNVKAVILDMFGAGTDTSSATIEWAISELIRCPRAMEKVQTELRQALNGKERIQEEDIQELSYLKLVIKETLRLHPPLPLVMPRECREPCVLAGYEIPTKTKLIVNVFAINRDPEYWKDAETFMPERFENSPINIMGSEYEYLPFGAGRRMCPGAALGLANVELPLAHILYYFNWKLPNGARLDELDMSECFGATVQRKSELLLVPTAYKTANNSA

SEQ ID NO: 50 - protein, 486 aa, Hyoscyamus muticus
FLLRKWKNSNSQSKKLPPGPWKLPLLGSMLHMVGGLPHHVLRDLAKKYGPLMHLQLGEVSAVVVTSPDMAKEVLKTHDIAFASRPKLLAPEIVCYNRSDIAFCPYGDYWRQMRKICVLEVLSAKNVRSFSSIRRDEVLRLVNFVRSSTSEPVNFTERLFLFTSSMTCRSAFGKVFKEQETFIQLIKEVIGLAGGFDVADIFPSLKFLHVLTGMEGKIMKAHHKVDAIVEDVINEHKKNLAMGKTNGALGGEDLIDVLLRLMNDGGLQFPITNDNIKAIIFDMFAAGTETSSSTLVWAMVQMMRNPTILAKAQAEVREAFKGKETFDENDVEELKYLKLVIKETLRLHPPVPLLVPRECREETEINGYTIPVKTKVMVNVWALGRDPKYWDDADNFKPERFEQCSVDFIGNNFEYLPFGGGRRICPGISFGLANVYLPLAQLLYHFDWKLPTGMEPKDLDLTELVGVTAARKSDLMLVATPYQPSRE

SEQ ID NO: 51 - protein, 469 aa, Lactuca sativa
KLATRPKSTKKQLPEASRLPIIGHMHHLIGTMPHRGVMDLARKHGSLMHLQLGEVSTIVVSSPKWAKEILTTYDITFANRPETLTGEIIAYHNTDIVLAPYGEYWRQLRKLCTLELLSVKKVKSFQSIREEECWNLVKEVKESGSGKPINLSESIFTMIATILSRAAFGKGIKDQREFTEIVKEILRQTGGFDVADIFPSKKFLHHLSGKRARLTSIHKKLDNLINNIVAEHHVSTSSKANETLLDVLLRLKDSAEFPLTADNVKAIILDMFGAGTDTSSATVEWAISELIRCPRAMEKVQAELRQALNGKEKIQEEDIQDLAYLNLVIRETLRLHPPLPLVMPRECREPVNLAGYEIANKTKLIVNVFAINRDPEYWKDAEAFIPERFENNPNNIMGADYEYLPFGAGRRMCPGAALGLANVQLPLANILYHFNWKLPNGASHDQLDMTESFGATVQRKTELLLVPSF

SEQ ID NO: 52 - protein, 488 aa, Nicotiani tabacum
FLLRKWKNSNSQSKKLPPGPWKIPILGSMLHMIGGEPHHVLRDLAKKYGPLMHLQLGEISAVVVTSRDMAKEVLKTHDVVFASRPKIVAMDIICYNQSDIAFSPYGDHWRQMRKICVMELLNAKNVRSFSSIRRDEVVRLIDSIRSDSSSGELVNFTQRIIWFASSMTCRSAFGQVLKGQDIFAKKIREVIGLAEGFDVVDIFPTYKFLHVLSGMKRKLLNAHLKVDAIVEDVINEHKKNLAAGKSNGALGGEDLIDVLLRLMNDTSLQFPITNDNIKAVIVDMFAAGTETSSTTTVWAMAEMMKNPSVFTKAQAEVREAFRDKVSFDENDVEELKYLKLVIKETLRLHPPSPLLVPRECREDTDINGYTIPAKTKVMVNVWALGRDPKYWDDAESFKPERFEQCSVDFFGNNFEFLPFGGGRRICPGMSFGLANLYLPLAQLLYHFDWKLPTGIMPRDLDLTELSGITIARKGGLYLNATPYQPSRE

SEQ ID NO: 53 - protein, 496 aa, Citrus x paradisi
WVWLRPKKLEKFLRQQGLKGNSYRLLFGDLKENSIELKEAKARPLSLDDDIAIRVNPFLHKLVNDYGKNSFMWFGPTPRVNIMNPDQIKAIFTKINDFQKVNSIPLARLLIVGLATLEGEKWAKHRKLINPAFHQEKLKLMLPAFYLSCIEIITKWEKQMSVEGSSELDVWPYLANLTSDVISRTAFGSSYEEGRRIFQLQAELAELTMQVFRSVHIPGWRFLPTKRNRRMKEIDKEIRASLMGIIKNREKAMRAGEAANNDLLGILMETSFREIEEHGNNKNVGFSMNDVIEECKLFYFAGQETTSVLLNWTMVLLSKHQDWQERARQEVLQVFGNNKPDYDGLNHLKIVQMILYEVLRLYPPVTVLSRAVFKETKLGNLTLPAGVQIGLPMILVHQDPELWGDDAVEFKPERFAEGISKAAKNQVSYFPFALGPRICVGQNFALVEAKMATAMILQNYSFELSPSYVHAPTAVPTLHPELGTQLILRKLWCKNN

SEQ ID NO: 54 - protein, 472 aa, Artemesia annua
FVYKFATRSKSTKKSLPEPWRLPIIGHMHHLIGTTPHRGVRDLARKYGSLMHLQLGEVPTIVVSSPKWAKEILTTYDITFANRPETLTGEIVLYHNTDVVLAPYGEYWRQLRKICTLELLSVKKVKSFQSLREEECWNLVQEIKASGSGRPVNLSENVFKLIATILSRAAFGKGIKDQKELTEIVKEILRQTGGFDVADIFPSKKFLHHLSGKRARLTSLRKKIDNLIDNLVAEHTVNTSSKTNETLLDVLLRLKDSAEFPLTSDNIKAIILDMFGAGTDTSSSTIEWAISELIKCPKAMEKVQAELRKALNGKEKIHEEDIQELSYLNMVIKETLRLHPPLPLVLPRECRQPVNLAGYNIPNKTKLIVNVFAINRDPEYWKDAEAFIPERFENSSATVMGAEYEYLPFGAGRRMCPGAALGLANVQLPLANILYHFNWKLPNGVSYDQIDMTESSGATMQRKTELLLVPSF

SEQ ID NO: 55 - protein, 488 aa, Arabidopsis thaliana
FFFKKLLSFSRKNMSEVSTLPSVPVVPGFPVIGNLLQLKEKKPHKTFTRWSEIYGPIYSIKMGSSSLIVLNSTETAKEAMVTRFSSISTRKLSNALTVLTCDKSMVATSDYDDFHKLVKRCLLNGLLGANAQKRKRHYRDALIENVSSKLHAHARDHPQEPVNFRAIFEHELFGVALKQAFGKDVESIYVKELGVTLSKDEIFKVLVHDMMEGAIDVDWRDFFPYLKWIPNKSFEARIQQKHKRRLAVMNALIQDRLKQNGSESDDDCYLNFLMSEAKTLTKEQIAILVWETIIETADTTLVTTEWAIYELAKHPSVQDRLCKEIQNVCGGEKFKEEQLSQVPYLNGVFHETLRKYSPAPLVPIRYAHEDTQIGGYHVPAGSEIAINIYGCNMDKKRWERPEDWWPERFLDDGKYETSDLHKTMAFGAGKRVCAGALQASLMAGIAIGRLVQEFEWKLRDGEEENVDTYGLTSQKLYPLMAIINPRRS

SEQ ID NO: 56 - protein, 483 aa, Stevia rebaudiana
WYLKSYTSARRSQSNHLPRVPEVPGVPLLGNLLQLKEKKPYMTFTRWAATYGPIYSIKTGATSMVVVSSNEIAKEALVTRFQSISTRNLSKALKVLTADKTMVAMSDYDDYHKTVKRHILTAVLGPNAQKKHRIHRDIMMDNISTQLHEFVKNNPEQEEVDLRKIFQSELFGLAMRQALGKDVESLYVEDLKITMNRDEIFQVLVVDPMMGAIDVDWRDFFPYLKWVPNKKFENTIQQMYIRREAVMKSLIKEHKKRIASGEKLNSYIDYLLSEAQTLTDQQLLMSLWEPIIESSDTTMVTTEWAMYELAKNPKLQDRLYRDIKSVCGSEKITEEHLSQLPYITAIFHETLRRHSPVPIIPLRHVHEDTVLGGYHVPAGTELAVNIYGCNMDKNVWENPEEWNPERFMKENETIDFQKTMAFGGGKRVCAGSLQALLTASIGIGRMVQEFEWKLKDMTQEEVNTIGLTTQMLRPLRAIIKPRI

SEQ ID NO: 57 - protein, 494 aa, Physcomitrella patens
FVARTCLRNKKRLPPAIPGGLPVLGNLLQLTEKKPHRTFTAWSKEHGPIFTIKVGSVPQAVVNNSEIAKEVLVTKFASISKRQMPMALRVLTRDKTMVAMSDYGEEHRMLKKLVMTNLLGPTTQNKNRSLRDDALIGMIEGVLAELKASPTSPKVVNVRDYVQRSLFPFALQQVFGYIPDQVEVLELGTCVSTWDMFDALVVAPLSAVINVDWRDFFPALRWIPNRSVEDLVRTVDFKRNSIMKALIRAQRMRLANLKEPPRCYADIALTEATHLTEKQLEMSLWEPIIESADTTLVTSEWAMYEIAKNPDCQDRLYREIVSVAGTERMVTEDDLPNMPYLGAIIKETLRKYTPVPLIPSRFVEEDITLGGYDIPKGYQILVNLFAIANDPAVWSNPEKWDPERMLANKKVDMGFRDFSLMPFGAGKRMCAGITQAMFIIPMNVAALVQHCEWRLSPQEISNINNKIEDVVYLTTHKLSPLSCEATPRISHRLP

SEQ ID NO: 58 - protein, 381 aa, Pleurotus sapidus
MGKLHPLAIIPDYKGSMAASVTIFNKRTNPLDISVNQANDWPWRYAKTCVLSSDWALHEMIIHLNNTHLVEEAVIVAAQRKLSPSHIVFRLLEPHWVVTLSLNALARSVLIPEVIVPIAGFSAPHIFQFIRESFTNFDWKSLYVPADLESRGFPVDQLNSPKFHNYAYARDINDMWTTLKKFVSSVLQDAQYYPDDASVAGDTQIQAWCDEMRSGMGAGMTNFPESITTVDDLVNMVTMCIHIAAPQHTAVNYLQQYYQTFVSNKPSALFSPLPTSIAQLQKYTESDLMAALPLNAKRQWLLMAQIPYLLSMQVQEDENIVTYAANASTDKDPIIASAGRQLAADLKKLAAVFLVNSAQLDDQNTPYDVLAPEQLANAIVI

SEQ ID NO: 59 - protein, 475 aa, Cichorium intybus
LLTRTTSKKNLLPEPWRLPIIGHMHHLIGTMPHRGVMELARKHGSLMHLQLGEVSTIVVSSPRWAKEVLTTYDITFANRPETLTGEIVAYHNTDIVLAPYGEYWRQLRKLCTLELLSNKKVKSFQSLREEECWNLVKDIRSTGQGSPINLSENIFKMIATILSRAAFGKGIKDQMKFTELVKEILRLTGGFDVADIFPSKKLLHHLSGKRAKLTNIHNKLDNLINNIIAEHPGNRTSSSQETLLDVLLRLKESAEFPLTADNVKAVILDMFGAGTDTSSATIEWAISELIRCPRAMEKVQTELRQALNGKERIQEEDLQELNYLKLVIKETLRLHPPLPLVMPRECREPCVLGGYDIPSKTKLIVNVFAINRDPEYWKDAETFMPERFENSPITVMGSEYEYLPFGAGRRMCPGAALGLANVELPLAHILYFNWKLPNGKTFEDLDMTESFGATVQRKTELLLVPTDFQTLTAST

SEQ ID NO: 60 - protein, 468 aa, Helianthus annuus
LLTRPTSSKNRLPEPWRLPIIGHMHHLIGTMPHRGVMDLARKYGSLMHLQLGEVSAIVVSSPKWAKEILTTYDIPFANRPETLTGEIIAYHNTDIVLAPYGEYWRQLRKLCTLELLSVKKVKSFQSLREEECWNLVQEIKASGSGTPFNLSEGIFKVIATVLSRAAFGKGIKDQKQFTEIVKEILRETGGFDVADIFPSKKFLHHLSGKRGRLTSIHNKLDSLINNLVAEHTVSKSSKVNETLLDVLLRLKNSEEFPLTADNVKAIILDMFGAGTDTSSATVEWAISELIRCPRAMEKVQAELRQALNGKERIKEEEIQDLPYLNLVIRETLRLHPPLPLVMPRECRQAMNLAGYDVANKTKLIVNVFAINRDPEYWKDAESFNPERFENSNTTIMGADYEYLPFGAGRRMCPGSALGLANVQLPLANILYYFKWKLPNGASHDQLDMTESFGATVQRKTELMLVPSF